European Patent Specification EP 4 514 842 B1, published March 25, 2026. Title: SARS-COV-2 ANTIBODIES AND METHODS OF USING THE SAME. Applicant: AstraZeneca UK Limited. Application WO. The sequence listing filed with the application follows.

SEQUENCE LISTING (82 sequences)

SEQ ID NO: 1 - protein, 1273 aa, synthetic construct
MFVFLVLLPLVSSQCVNLTTRTQLPPAYTNSFTRGVYYPDKVFRSSVLHSTQDLFLPFFSNVTWFHAIHVSGTNGTKRFDNPVLPFNDGVYFASTEKSNIIRGWIFGTTLDSKTQSLLIVNNATNVVIKVCEFQFCNDPFLGVYYHKNNKSWMESEFRVYSSANNCTFEYVSQPFLMDLEGKQGNFKNLREFVFKNIDGYFKIYSKHTPINLVRDLPQGFSALEPLVDLPIGINITRFQTLLALHRSYLTPGDSSSGWTAGAAAYYVGYLQPRTFLLKYNENGTITDAVDCALDPLSETKCTLKSFTVEKGIYQTSNFRVQPTESIVRFPNITNLCPFGEVFNATRFASVYAWNRKRISNCVADYSVLYNSASFSTFKCYGVSPTKLNDLCFTNVYADSFVIRGDEVRQIAPGQTGKIADYNYKLPDDFTGCVIAWNSNNLDSKVGGNYNYLYRLFRKSNLKPFERDISTEIYQAGSTPCNGVEGFNCYFPLQSYGFQPTNGVGYQPYRVVVLSFELLHAPATVCGPKKSTNLVKNKCVNFNFNGLTGTGVLTESNKKFLPFQQFGRDIADTTDAVRDPQTLEILDITPCSFGGVSVITPGTNTSNQVAVLYQDVNCTEVPVAIHADQLTPTWRVYSTGSNVFQTRAGCLIGAEHVNNSYECDIPIGAGICASYQTQTNSPRRARSVASQSIIAYTMSLGAENSVAYSNNSIAIPTNFTISVTTEILPVSMTKTSVDCTMYICGDSTECSNLLLQYGSFCTQLNRALTGIAVEQDKNTQEVFAQVKQIYKTPPIKDFGGFNFSQILPDPSKPSKRSFIEDLLFNKVTLADAGFIKQYGDCLGDIAARDLICAQKFNGLTVLPPLLTDEMIAQYTSALLAGTITSGWTFGAGAALQIPFAMQMAYRFNGIGVTQNVLYENQKLIANQFNSAIGKIQDSLSSTASALGKLQDVVNQNAQALNTLVKQLSSNFGAISSVLNDILSRLDKVEAEVQIDRLITGRLQSLQTYVTQQLIRAAEIRASANLAATKMSECVLGQSKRVDFCGKGYHLMSFPQSAPHGVVFLHVTYVPAQEKNFTTAPAICHDGKAHFPREGVFVSNGTHWFVTQRNFYEPQIITTDNTFVSGNCDVVIGIVNNTVYDPLQPELDSFKEELDKYFKNHTSPDVDLGDISGINASVVNIQKEIDRLNEVAKNLNESLIDLQELGKYEQYIKWPWYIWLGFIAGLIAIVMVTIMLCCMTSCCSCLKGCCSCGSCCKFDEDDSEPVLKGVKLHYT

SEQ ID NO: 2 - protein, 5 aa, synthetic construct
  source 1..5: note = CDR1
TSAVQ

SEQ ID NO: 3 - protein, 17 aa, synthetic construct
  source 1..17: note = CDR2
WIAVGSGNTNYAQKFQD

SEQ ID NO: 4 - protein, 14 aa, synthetic construct
  source 1..14: note = CDR3
PHCDRTSCHDGFDI

SEQ ID NO: 5 - protein, 12 aa, synthetic construct
  source 1..12: note = CDR1
RASQSVRSSYLA

SEQ ID NO: 6 - protein, 7 aa, synthetic construct
  source 1..7: note = CDR2
GASRRGT

SEQ ID NO: 7 - protein, 9 aa, synthetic construct
  source 1..9: note = CDR3
QQYGSSPWT

SEQ ID NO: 8 - protein, 5 aa, synthetic construct
  source 1..5: note = CDR1
TYVFT

SEQ ID NO: 9 - protein, 17 aa, synthetic construct
  source 1..17: note = CDR2
GIIPFFGTADYAQKFQG

SEQ ID NO: 10 - protein, 9 aa, synthetic construct
  source 1..9: note = CDR3
LSQWDLLPM

SEQ ID NO: 11 - protein, 12 aa, synthetic construct
  source 1..12: note = CDR1
RASQSFTSSYLA

SEQ ID NO: 12 - protein, 11 aa, synthetic construct
  source 1..11: note = CDR3
QQYGTSPRMYT

SEQ ID NO: 13 - protein, 7 aa, synthetic construct
  source 1..7: note = CDR1
SSNHYWV

SEQ ID NO: 14 - protein, 16 aa, synthetic construct
  source 1..16: note = CDR2
SMYYSGSTAYNPSLTN

SEQ ID NO: 15 - protein, 16 aa, synthetic construct
  source 1..16: note = CDR3
QIGPKRPSQVADWFDP

SEQ ID NO: 16 - protein, 11 aa, synthetic construct
  source 1..11: note = CDR1
RASQGISSYLA

SEQ ID NO: 17 - protein, 7 aa, synthetic construct
  source 1..7: note = CDR2
AASTLQS

SEQ ID NO: 18 - protein, 9 aa, synthetic construct
  source 1..9: note = CDR3
QQLNSYPLT

SEQ ID NO: 19 - protein, 16 aa, synthetic construct
  source 1..16: note = CDR3
QIGPKRPSQVADWFEP

SEQ ID NO: 20 - protein, 5 aa, synthetic construct
  source 1..5: note = CDR1
SYAIN

SEQ ID NO: 21 - protein, 17 aa, synthetic construct
  source 1..17: note = CDR2
GIIPIFRTPHYAQKFQG

SEQ ID NO: 22 - protein, 22 aa, synthetic construct
  source 1..22: note = CDR3
PSCGGDCPQYLKSSKLDWYFDL

SEQ ID NO: 23 - protein, 12 aa, synthetic construct
  source 1..12: note = CDR1
RASQSVSSTYLA

SEQ ID NO: 24 - protein, 9 aa, synthetic construct
  source 1..9: note = CDR3
QHYGSSPLT

SEQ ID NO: 25 - protein, 5 aa, synthetic construct
  source 1..5: note = CDR1
RNYMS

SEQ ID NO: 26 - protein, 16 aa, synthetic construct
  source 1..16: note = CDR2
VIYSGGSTFYADSVKG

SEQ ID NO: 27 - protein, 10 aa, synthetic construct
  source 1..10: note = CDR3
DLDVVGGTDY

SEQ ID NO: 28 - protein, 12 aa, synthetic construct
  source 1..12: note = CDR1
RASQSVSSSYLA

SEQ ID NO: 29 - protein, 10 aa, synthetic construct
  source 1..10: note = CDR3
QQYGSSPGYT

SEQ ID NO: 30 - protein, 10 aa, synthetic construct
  source 1..10: note = CDR3
DLEVVGGTDY

SEQ ID NO: 31 - protein, 5 aa, synthetic construct
  source 1..5: note = CDR1
DYAIH

SEQ ID NO: 32 - protein, 17 aa, synthetic construct
  source 1..17: note = CDR2
SISWDSGSIGYADSVKG

SEQ ID NO: 33 - protein, 16 aa, synthetic construct
  source 1..16: note = CDR3
GAFPGYSSGWYYGLDV

SEQ ID NO: 34 - protein, 14 aa, synthetic construct
  source 1..14: note = CDR1
TGTSSDVGGYNYVS

SEQ ID NO: 35 - protein, 7 aa, synthetic construct
  source 1..7: note = CDR2
EVSKRPS

SEQ ID NO: 36 - protein, 9 aa, synthetic construct
  source 1..9: note = CDR3
SSYAGNKGV

SEQ ID NO: 37 - protein, 16 aa, synthetic construct
  source 1..16: note = CDR3
GAFPGYSSGWYYGLEV

SEQ ID NO: 38 - protein, 123 aa, synthetic construct
  source 1..123: note = H Variable Sequence Region
QVQLVESGPEMKKPGTSVKVSCKASGFTFITSAVQWVRQARGQRLEWMGWIAVGSGNTNYAQKFQDRVTINRDMSTSTAYMELSSLRSEDTAVYYCAAPHCDRTSCHDGFDIWGQGTMVTVSS

SEQ ID NO: 39 - protein, 108 aa, synthetic construct
  source 1..108: note = L Variable Sequence Region
DIVMTQSPGTLSLSPGERATLSCRASQSVRSSYLAWYQQKPGQAPRLLIYGASRRGTGIPDRFSGSGSGTDFTLTISRLEPEDFAVYYCQQYGSSPWTFGQGTKVEIK

SEQ ID NO: 40 - protein, 123 aa, synthetic construct
  source 1..123: note = H Variable Sequence Region
QVQLVQSGPEVKKPGTSVKVSCKASGFTFITSAVQWVRQARGQRLEWMGWIAVGSGNTNYAQKFQDRVTITRDMSTSTAYMELSSLRSEDTAVYYCAAPHCDRTSCHDGFDIWGQGTMVTVSS

SEQ ID NO: 41 - protein, 108 aa, synthetic construct
  source 1..108: note = L Variable Sequence Region
EIVMTQSPGTLSLSPGERATLSCRASQSVRSSYLAWYQQKPGQAPRLLIYGASRRGTGIPDRFSGSGSGTDFTLTISRLEPEDFAVYYCQQYGSSPWTFGGGTKVEIK

SEQ ID NO: 42 - protein, 118 aa, synthetic construct
  source 1..118: note = H Variable Sequence Region
EVQLVQSGAEVKKPGSSVKVSCKASRGTFNTYVFTWVRQAPGQGLEWMGGIIPFFGTADYAQKFQGRVTITADDSTSTAYMELSSLRSEDTAVYYCSRLSQWDLLPMWGQGTLVTVSS

SEQ ID NO: 43 - protein, 110 aa, synthetic construct
  source 1..110: note = L Variable Sequence Region
DIVMTQSPGTLSLSPGERATLSCRASQSFTSSYLAWYQQKPGQAPRLLIYGASSRATGIPDRFSGTGSGTDFTLTISRLEPEDFAVYYCQQYGTSPRMYTFGQGTKVDIK

SEQ ID NO: 44 - protein, 118 aa, synthetic construct
  source 1..118: note = H Variable Sequence Region
QVQLVQSGAEVKKPGSSVKVSCKASRGTFNTYVFTWVRQAPGQGLEWMGGIIPFFGTADYAQKFQGRVTITADESTSTAYMELSSLRSEDTAVYYCSRLSQWDLLPMWGQGTLVTVSS

SEQ ID NO: 45 - protein, 110 aa, synthetic construct
  source 1..110: note = L Variable Sequence Region
EIVMTQSPGTLSLSPGERATLSCRASQSFTSSYLAWYQQKPGQAPRLLIYGASSRATGIPDRFSGSGSGTDFTLTISRLEPEDFAVYYCQQYGTSPRMYTFGQGTKLEIK

SEQ ID NO: 46 - protein, 126 aa, synthetic construct
  source 1..126: note = H Variable Sequence Region
QVQLQESGPGLVKPSETLSLTCTVFGGSITSSNHYWVWIRQPPGKGLEWIGSMYYSGSTAYNPSLTNRVTISVDTSKNQFSLKLSSVTAADTAVYYCARQIGPKRPSQVADWFDPWGQGTLVTVSS

SEQ ID NO: 47 - protein, 107 aa, synthetic construct
  source 1..107: note = L Variable Sequence Region
DIQLTQSPSFLSASVGDRVTITCRASQGISSYLAWYQQKPGKAPKLLIYAASTLQSGVPSRFSGSGSGTEFTLTISSLQPEDFATYYCQQLNSYPLTFGGGTKVEIK

SEQ ID NO: 48 - protein, 126 aa, synthetic construct
  source 1..126: note = H Variable Sequence Region
QVQLQESGPGLVKPSETLSLTCTVSGGSITSSNHYWVWIRQPPGKGLEWIGSMYYSGSTAYNPSLTNRVTISVDTSKNQFSLKLSSVTAADTAVYYCARQIGPKRPSQVADWFDPWGQGTLVTVSS

SEQ ID NO: 49 - protein, 126 aa, synthetic construct
  source 1..126: note = H Variable Sequence Region
QVQLQESGPGLVKPSETLSLTCTVSGGSITSSNHYWVWIRQPPGKGLEWIGSMYYSGSTAYNPSLTNRVTISVDTSKNQFSLKLSSVTAADTAVYYCARQIGPKRPSQVADWFEPWGQGTLVTVSS

SEQ ID NO: 50 - protein, 131 aa, synthetic construct
  source 1..131: note = H Variable Sequence Region
EVQLVESGAEVKKPGSSVKVSCKASGGTFSSYAINWVRQAPGQGLEWMGGIIPIFRTPHYAQKFQGRVTITADESTGTAYMELSSLRSEDTAVYYCASPSCGGDCPQYLKSSKLDWYFDLWGRGTLVTVSS

SEQ ID NO: 51 - protein, 108 aa, synthetic construct
  source 1..108: note = L Variable Sequence Region
VIWMTQSPGTLSLSPGERATLSCRASQSVSSTYLAWYQQKPGQAPRLLIYGASSRATGIPDRFSGSGSGTDFTLTISRLEPEDFAVYYCQHYGSSPLTFGQGTRLEIK

SEQ ID NO: 52 - protein, 131 aa, synthetic construct
  source 1..131: note = H Variable Sequence Region
QVQLVQSGAEVKKPGSSVKVSCKASGGTFSSYAINWVRQAPGQGLEWMGGIIPIFRTPHYAQKFQGRVTITADESTSTAYMELSSLRSEDTAVYYCASPSCGGDCPQYLKSSKLDWYFDLWGRGTLVTVSS

SEQ ID NO: 53 - protein, 108 aa, synthetic construct
  source 1..108: note = L Variable Sequence Region
EIVMTQSPGTLSLSPGERATLSCRASQSVSSTYLAWYQQKPGQAPRLLIYGASSRATGIPDRFSGSGSGTDFTLTISRLEPEDFAVYYCQHYGSSPLTFGQGTRLEIK

SEQ ID NO: 54 - protein, 118 aa, synthetic construct
  source 1..118: note = H Variable Sequence Region
EVQLVESGGGLIQPGGSLRLSCAASEIIVSRNYMSWVRQAPGKGLEWVSVIYSGGSTFYADSVKGRFTISRDNSKNTLYLQMNSLRAEDTAVYYCARDLDVVGGTDYWGQGTLVTVSS

SEQ ID NO: 55 - protein, 109 aa, synthetic construct
  source 1..109: note = L Variable Sequence Region
EIVLTQSPGTLSLSPGERATLSCRASQSVSSSYLAWYQQKPGQAPRLLIYGASSRATGIPDRFSGSGSGTDFTLTISRLEPEDFAVYYCQQYGSSPGYTFGQGTKVDIK

SEQ ID NO: 56 - protein, 118 aa, synthetic construct
  source 1..118: note = H Variable Sequence Region
EVQLVETGGGLIQPGGSLRLSCAASEIIVSRNYMSWVRQAPGKGLEWVSVIYSGGSTFYADSVKGRFTISRDNSKNTLYLQMNSLRAEDTAVYYCARDLDVVGGTDYWGQGTLVTVSS

SEQ ID NO: 57 - protein, 109 aa, synthetic construct
  source 1..109: note = L Variable Sequence Region
EIVLTQSPGTLSLSPGERATLSCRASQSVSSSYLAWYQQKPGQAPRLLIYGASSRATGIPDRFSGSGSGTDFTLTISRLEPEDFAVYYCQQYGSSPGYTFGPGTKVDIK

SEQ ID NO: 58 - protein, 117 aa, synthetic construct
  source 1..117: note = H Variable Sequence Region
EVQLVETGGGLIQPGGSLRLSCAASEIIVSRNYMSWVRQAPGKGLEWVSVIYSGGSTFYADSVKGRFTISRDNSKNLYLQMNSLRAEDTAVYYCARDLEVVGGTDYWGQGTLVTVSS

SEQ ID NO: 59 - protein, 118 aa, synthetic construct
  source 1..118: note = H Variable Sequence Region
EVQLVESGGGLIQPGGSLRLSCAASEIIVSRNYMSWVRQAPGKGLEWVSVIYSGGSTFYADSVKGRFTISRDNSKNTLYLQMNSLRAEDTAVYYCARDLEVVGGTDYWGQGTLVTVSS

SEQ ID NO: 60 - protein, 125 aa, synthetic construct
  source 1..125: note = H Variable Sequence Region
EVQLLETGGGLVQPGRSLRLSCAASGFPFDDYAIHWVRLAPGKGLEWVSSISWDSGSIGYADSVKGRFTISRDNAKNSLYLQMNSLRAEDTALYYCAKGAFPGYSSGWYYGLDVWGQGATVTVSS

SEQ ID NO: 61 - protein, 109 aa, synthetic construct
  source 1..109: note = L Variable Sequence Region
QSVVTQPPSASGSLGQSVTISCTGTSSDVGGYNYVSWYQQHPGKAPKLMIFEVSKRPSGVPDRFSGSKSGNTASLTVSGLQAEDEADYYCSSYAGNKGVFGGGTKLTVL

SEQ ID NO: 62 - protein, 125 aa, synthetic construct
  source 1..125: note = H Variable Sequence Region
EVQLVESGGGLVQPGRSLRLSCAASGFPFDDYAIHWVRLAPGKGLEWVSSISWDSGSIGYADSVKGRFTISRDNAKNSLYLQMNSLRAEDTALYYCAKGAFPGYSSGWYYGLDVWGQGTTVTVSS

SEQ ID NO: 63 - protein, 125 aa, synthetic construct
  source 1..125: note = H Variable Sequence Region
EVQLVESGGGLVQPGRSLRLSCAASGFPFDDYAIHWVRLAPGKGLEWVSSISWDSGSIGYADSVKGRFTISRDNAKNSLYLQMNSLRAEDTALYYCAKGAFPGYSSGWYYGLEVWGQGTTVTVSS

SEQ ID NO: 64 - protein, 109 aa, synthetic construct
  source 1..109: note = L Variable Sequence Region
QSAVTQPASVSGSPGQSITISCTGTSSDVGGYNYVSWYQQHPGKAPKLMIFEVSKRPSGVSNRFSGSKSGNTASLTISGLQAEDEADYYCSSYAGNKGVFGSGTKVTVL

SEQ ID NO: 65 - protein, 106 aa, synthetic construct
GQPKAAPSVTLFPPSSEELQANKATLVCLISDFYPGAVTVAWKADSSPVKAGVETTTPSKQSNNKYAASSYLSLTPEQWKSHRSYSCQVTHEGSTVEKTVAPTECS

SEQ ID NO: 66 - protein, 330 aa, synthetic construct
ASTKGPSVFPLAPSSKSTSGGTAALGCLVKDYFPEPVTVSWNSGALTSGVHTFPAVLQSSGLYSLSSVVTVPSSSLGTQTYICNVNHKPSNTKVDKRVEPKSCDKTHTCPPCPAPEFEGGPSVFLFPPKPKDTLYITREPEVTCVVVDVSHEDPEVKFNWYVDGVEVHNAKTKPREEQYNSTYRVVSVLTVLHQDWLNGKEYKCKVSNKALPASIEKTISKAKGQPREPQVYTLPPSREEMTKNQVSLTCLVKGFYPSDIAVEWESNGQPENNYKTTPPVLDSDGSFFLYSKLTVDKSRWQQGNVFSCSVMHEALHNHYTQKSLSLSPGK

SEQ ID NO: 67 - protein, 7 aa, synthetic construct
  source 1..7: note = CDR2
GASSRAT

SEQ ID NO: 68 - protein, 123 aa, synthetic construct
  source 1..123: note = H Variable Sequence Region
QMQLVQSGPEVKKPGTSVKVSCKASGFTFMSSAVQWVRQARGQRLEWIGWIVIGSGNTNYAQKFQERVTITRDMSTSTAYMELSSLRSEDTAVYYCAAPYCSSISCNDGFDIWGQGTMVTVSS

SEQ ID NO: 69 - protein, 8 aa, synthetic construct
  source 1..8: note = CDR1
GFTFMSSA

SEQ ID NO: 70 - protein, 8 aa, synthetic construct
  source 1..8: note = CDR2
IVIGSGNT

SEQ ID NO: 71 - protein, 16 aa, synthetic construct
  source 1..16: note = CDR3
AAPYCSSISCNDGFDI

SEQ ID NO: 72 - protein, 109 aa, synthetic construct
  source 1..109: note = L Variable Sequence Region
EIVLTQSPGTLSLSPGERATLSCRASQSVSSSYLAWYQQKPGQAPRLLIYGASSRATGIPDRFSGSGSGTDFTLTISRLEPEDFAVYYCQHYGSSRGWTFGQGTKVEIK

SEQ ID NO: 73 - protein, 7 aa, synthetic construct
  source 1..7: note = CDR1
QSVSSSY

SEQ ID NO: 74 - skipped

SEQ ID NO: 75 - protein, 10 aa, synthetic construct
  source 1..10: note = CDR3
QHYGSSRGWT

SEQ ID NO: 76 - protein, 461 aa, synthetic construct
  source 1..461: note = H
EVQLVESGGGLVKPGGSLRLSCAASGFTFRDVWMSWVRQAPGKGLEWVGRIKSKIDGGTTDYAAPVKGRFTISRDDSKNTLYLQMNSLKTEDTAVYYCTTAGSYYYDTVGPGLPEGKFDYWGQGTLVTVSSASTKGPSVFPLAPSSKSTSGGTAALGCLVKDYFPEPVTVSWNSGALTSGVHTFPAVLQSSGLYSLSSVVTVPSSSLGTQTYICNVNHKPSNTKVDKRVEPKSCDKTHTCPPCPAPEFEGGPSVFLFPPKPKDTLYITREPEVTCVVVDVSHEDPEVKFNWYVDGVEVHNAKTKPREEQYNSTYRVVSVLTVLHQDWLNGKEYKCKVSNKALPASIEKTISKAKGQPREPQVYTLPPSREEMTKNQVSLTCLVKGFYPSDIAVEWESNGQPENNYKTTPPVLDSDGSFFLYSKLTVDKSRWQQGNVFSCSVMHEALHNHYTQKSLSLSPGK

SEQ ID NO: 77 - protein, 219 aa, synthetic construct
  source 1..219: note = L
DIVMTQSPDSLAVSLGERATINCKSSQSVLYSSNNKNYLAWYQQKPGQPPKLLMYWASTRESGVPDRFSGSGSGAEFTLTISSLQAEDVAIYYCQQYYSTLTFGGGTKVEIKRTVAAPSVFIFPPSDEQLKSGTASVVCLLNNFYPREAKVQWKVDNALQSGNSQESVTEQDSKDSTYSLSSTLTLSKADYEKHKVYACEVTHQGLSSPVTKSFNRGEC

SEQ ID NO: 78 - protein, 14 aa, synthetic construct
NNLDSKVGGNYNYL

SEQ ID NO: 79 - protein, 16 aa, synthetic construct
EGFNCYFPLQSYGFQP

SEQ ID NO: 80 - protein, 19 aa, synthetic construct
RGDEVRQIAPGQTGKIADY

SEQ ID NO: 81 - protein, 7 aa, synthetic construct
YRLFRKS

SEQ ID NO: 82 - protein, 17 aa, synthetic construct
YQAGSTPCNGVEGFNCY